European Patent Specification EP 3 988 123 B1, published February 26, 2025. Title: Antibody-Coupled Cyclic Peptide Tyrosine Tyrosine Compounds as Modulators of Neuropeptide Y Receptors. Applicant: Janssen Pharmaceutica NV. The sequence listing filed with the application follows.

SEQUENCE LISTING (156 sequences)

SEQ ID NO: 1 - protein, 35 aa, Artificial Sequence
  Cyclic PYY Peptide Compound
  Ala (1)..(1): Ala with chemical modification as described in the specification
  Lys (10)..(10): Lys with chemical modification as described in the specification
  Cys (30)..(30): Cys, wherein Cys is a homocysteine with chemical modification as described in the specification
  Arg (34)..(34): Arg with chemical modification as described in the specification
AIKPEAPGEKASPEELNRYYASLRHYLNLCTRQRY

SEQ ID NO: 2 - protein, 34 aa, Artificial Sequence
  Cyclic PYY Peptide Compound
  Ile (1)..(1): Ile with chemical modification as described in the specification
  Cys (29)..(29): Cyse, wherein Cys is homocysteine with chemical modification as described in the specification
IKPEAPGEDASPEELNRYYASLRHYLNLCTRQRY

SEQ ID NO: 3 - protein, 34 aa, Artificial Sequence
  Cyclic PYY Peptide Compound
  Ile (1)..(1): Ile with the chemical modification as described in the specification
  Leu (29)..(29): Leu, wherien Leu is a norleucine with the chemical modification as described in the specification
IKPEAPGEDASPEELNRYYASLRHYLNLLTRQRY

SEQ ID NO: 4 - protein, 34 aa, Artificial Sequence
  Cyclic PYY Peptide Compound
  Ile (1)..(1): Ile with the chemical modification as described in the specification
  Lys (9)..(9): Lys with the chemical modification as described in the specification
  Cys (29)..(29): Cys, wherein cys is a homocysteine with the chemical modification as described in the specification
IKPEAPGEKASPEELNRYYASLRHYLNLCTRQRY

SEQ ID NO: 5 - protein, 34 aa, Artificial Sequence; identical to SEQ ID NO: 4
  Cyclic PYY Peptide Compound
  Ile (1)..(1): Ile with the chemical modification as described in the specification
  Lys (9)..(9): Lys with the chemical modification as described in the specification
  Cys (29)..(29): Cys, wherein cys is homocysteine with the chemical modification as described in the specification

SEQ ID NO: 6 - protein, 34 aa, Artificial Sequence
  Cyclic PYY Peptide Compound
  Ile (1)..(1): Ile with the chemical modification as described in the specification
  Lys (9)..(9): Lys with the chemical modification as described in the specification
  Leu (29)..(29): Leu, wherein the leu is norleucine with the chemical modification as described in the specification
IKPEAPGEKASPEELNRYYASLRHYLNLLTRQRY

SEQ ID NO: 7 - protein, 34 aa, Artificial Sequence
  Cyclic PYY Peptide Compound
  Ile (1)..(1): Ile with the chemical modification as described in the specification
  Lys (7)..(7): Lys with the chemical modification as described in the specification
  Cys (29)..(29): Cys, wherein cys is homocysteine with the chemical modification as described in the specification
IKPEAPKEDASPEELNRYYASLRHYLNLCTRQRY

SEQ ID NO: 8 - protein, 34 aa, Artificial Sequence
  Cyclic PYY Peptide Compound
  Ile (1)..(1): Ile with the chemical modification as described in the specification
  Lys (28)..(28): Lys with the chemical modification as described in the specification
  Cys (29)..(29): Cys, wherein cys is homocysteine with the chemical modification as described in the specification
IKPEAPGEDASPEELNRYYASLRHYLNKCTRQRY

SEQ ID NO: 9 - protein, 34 aa, Artificial Sequence; identical to SEQ ID NO: 2
  Cyclic PYY Peptide Compound
  Ile (1)..(1): Ile with the chemical modification as described in the specification
  Cys (29)..(29): Cys, wherein cys is a homocysteine with the chemical modification as described in the specification
  Arg (33)..(33): Arg with the chemical modification as described in the specification

SEQ ID NO: 10 - protein, 35 aa, Artificial Sequence
  Cyclic PYY Peptide Compound
  Ile (1)..(1): Ile with the chemical modification as described in the specification
  Lys (28)..(28): Lys with the chemical modification as described in the specification
  Cys (29)..(29): Cys, wherein cys is homocysteine with the chemical modification as described in the specification
IKPEAPGEDASPEELNRYYASLRHYLNLKCTRQRY

SEQ ID NO: 11 - protein, 35 aa, Artificial Sequence; identical to SEQ ID NO: 10
  Cyclic PYY Peptide Compound
  Ile (1)..(1): Ile with the chemical modification as described in the specification
  Lys (28)..(28): Lys with the chemical modification as described in the specification
  Cys (29)..(29): Cys, wherein cys is homocysteine with the chemical modification as described in the specification
  Arg (33)..(33): Arg with the chemical modification as described in the specification

SEQ ID NO: 12 - protein, 34 aa, Artificial Sequence; identical to SEQ ID NO: 2
  Cyclic PYY Peptide Compound
  Ile (1)..(1): Ile with the chemical modification as described in the specification
  Cys (29)..(29): Cys, wherein the cys is homocysteine with the chemical modification as described in the specification
  Arg (33)..(33): Arg with the chemical modification as described in the specification

SEQ ID NO: 13 - protein, 34 aa, Artificial Sequence; identical to SEQ ID NO: 8
  Cyclic PYY Peptide Compound
  Ile (1)..(1): Ile with the chemical modification as described in the specification
  Lys (28)..(28): Lys with the chemical modification as described in the specification
  Cys (29)..(29): Cys, wherein the cys is homocysteine with the chemical modification as described in the specification
  Arg (33)..(33): Arg with the chemical modification as described in the specification

SEQ ID NO: 14 - protein, 34 aa, Artificial Sequence; identical to SEQ ID NO: 8
  Cyclic PYY Peptide Compound
  Ile (1)..(1): Ile with the chemical modification as described in the specification
  Lys (28)..(28): Lys with the chemical modification as described in the specification
  Cys (29)..(29): Cys, wherein the cys is homocysteine with the chemical modification as described in the specification
  Arg (33)..(33): Arg with the chemical modification as described in the specification

SEQ ID NO: 15 - protein, 33 aa, Artificial Sequence
  Cyclic PYY Peptide Compound
  Lys (1)..(1): Lys with the chemical modification as described in the specification
  Lys (27)..(27): Lys with the chemical modification as described in the specification
  Cys (28)..(28): Cys, wherein cys is homocysteine with the chemical modification as described in the specification
KPEAPGEDASPEELNRYYASLRHYLNKCTRQRY

SEQ ID NO: 16 - protein, 33 aa, Artificial Sequence; identical to SEQ ID NO: 15
  Cyclic PYY Peptide Compound
  Lys (1)..(1): Lys with the chemical modification as described in the specification
  Lys (27)..(27): Lys with the chemical modification as described in the specification
  Cys (28)..(28): Cys, wherein the cys is homocysteine with the chemical modification as described in the specification

SEQ ID NO: 17 - protein, 34 aa, Artificial Sequence
  Cyclic PYY Peptide Compound
  Ile (1)..(1): Ile with the chemical modification as described in the specification
  Lys (28)..(28): Lys with the chemical modification as described in the specification
  Cys (29)..(29): Cys, wherein the cys is a homocysteine with the chemical modification as described in the specification
IAPEAPGEDASPEELNRYYASLRHYLNKCTRQRY

SEQ ID NO: 18 - protein, 34 aa, Artificial Sequence
  Cyclic PYY Peptide Compound
  Ile (1)..(1): Ile with the chemical modification as described in the specification
  Lys (28)..(28): Lys with the chemical modification as described in the specification
  Cys (29)..(29): Cys, wherein cys is homocysteine with the chemical modification as described in the specification
IEPEAPGEDASPEELNRYYASLRHYLNKCTRQRY

SEQ ID NO: 19 - protein, 34 aa, Artificial Sequence; identical to SEQ ID NO: 8
  Cyclic PYY Peptide Compound
  Ile (1)..(1): Ile with the chemical modification as described in the specification
  Lys (28)..(28): Lys with the chemical modification as described in the specification
  Cys (29)..(29): Cys with the chemical modification as described in the specification
  Arg (33)..(33): Arg with the chemical modification as described in the specification

SEQ ID NO: 20 - protein, 34 aa, Artificial Sequence; identical to SEQ ID NO: 8
  Cyclic PYY Peptide Compound
  Ile (1)..(1): Ile with the chemical modification as described in the specification
  Lys (28)..(28): Lys with the chemical modification as described in the specification
  Cys (29)..(29): Cys with the chemical modification as described in the specification
  Arg (33)..(33): Arg with the chemical modification as described in the specification

SEQ ID NO: 21 - protein, 34 aa, Artificial Sequence
  Cyclic PYY Peptide Compound
  Ile (1)..(1): Ile with the chemical modification as described in the specification
  Lys (28)..(28): Lys with the chemical modification as described in the specification
  Cys (29)..(29): Cys, wherein cys is a homocysteine with the chemical modification as described in the specification
IAPEAPGEDASPEELNRYYASLRAYLNKCTRQRY

SEQ ID NO: 22 - protein, 34 aa, Artificial Sequence
  Cyclic PYY Peptide Compound
  Ile (1)..(1): Ile with the chemical modification as described in the specification
  Lys (28)..(28): Lys with the chemical modification as described in the specification
  Cys (29)..(29): Cys, wherein the cys is a homocysteine with the chemical modification as described in the specification
IEPEAPGEDASPEELNRYYASLRAYLNKCTRQRY

SEQ ID NO: 23 - protein, 34 aa, Artificial Sequence; identical to SEQ ID NO: 8
  Cyclic PYY Peptide Compound
  Ile (1)..(1): Ile with the chemical modification as described in the specification
  Lys (28)..(28): Lys with the chemical modification as described in the specification
  Cys (29)..(29): Cys, wherein cys is a homocysteine with the chemical modification as described in the specification
  Arg (33)..(33): Arg with the chemical modification as described in the specification

SEQ ID NO: 24 - protein, 34 aa, Artificial Sequence; identical to SEQ ID NO: 8
  Cyclic PYY Peptide Compound
  Ile (1)..(1): Ile with the chemical modification as described in the specification
  Lys (28)..(28): Lys with the chemical modification as described in the specification
  Cys (29)..(29): Cys, wherein cys is homocysteine with the chemical modification as described in the specification
  Arg (33)..(33): Arg with the chemical modification as described in the specification

SEQ ID NO: 25 - protein, 34 aa, Artificial Sequence; identical to SEQ ID NO: 8
  Cyclic PYY Peptide Compound
  Ile (1)..(1): Ile with the chemical modification as described in the specification
  Lys (28)..(28): Lys with the chemical modification as described in the specification
  Cys (29)..(29): Cys, wherein cys is a homocysteine with the chemical modification as described in the specification
  Arg (33)..(33): Arg with the chemical modification as described in the specification

SEQ ID NO: 26 - protein, 34 aa, Artificial Sequence; identical to SEQ ID NO: 8
  Cyclic PYY Peptide Compound
  Ile (1)..(1): Ile with the chemical modification described in the application
  Lys (28)..(28): Lys with the chemical modification described in the application
  Cys (29)..(29): Cys, wherein the cys is a homocysteine with the chemical modification described in the application
  Arg (33)..(33): Arg with the chemical modification described in the application

SEQ ID NO: 27 - protein, 34 aa, Artificial Sequence; identical to SEQ ID NO: 8
  Cyclic PYY Peptide Compound
  Ile (1)..(1): Ile with the chemical modification described in the specification
  Lys (28)..(28): Lys with the chemical modification described in the specification
  Cys (29)..(29): Cys, wherein the cys is homocysteine with the chemical modification described in the specification
  Arg (33)..(33): Arg with the chemical modification described in the specification

SEQ ID NO: 28 - protein, 33 aa, Artificial Sequence; identical to SEQ ID NO: 15
  Cyclic PYY Peptide Compound
  Lys (1)..(1): Lys with the chemical modification described in the specification
  Lys (27)..(27): Lys with the chemical modification described in the specification
  Cys (28)..(28): Cys, wherein the cys is a homocysteine with the chemical modification described in the specification
  Arg (32)..(32): Arg with the chemical modification described in the specification

SEQ ID NO: 29 - protein, 33 aa, Artificial Sequence; identical to SEQ ID NO: 15
  Cyclic PYY Peptide Compound
  Lys (1)..(1): Lys with the chemical modification described in the specification
  Lys (27)..(27): Lys with the chemical modification described in the specification
  Cys (28)..(28): Cys, wherein the cys is a homocysteine with the chemical modification described in the specification
  Arg (32)..(32): Arg with the chemical modification described in the specification

SEQ ID NO: 30 - protein, 33 aa, Artificial Sequence; identical to SEQ ID NO: 15
  Cyclic PYY Peptide Compound
  Lys (1)..(1): Lys with the chemical modification described in the specification
  Lys (27)..(27): Lys with the chemical modification described in the specification
  Cys (28)..(28): Cys with the chemical modification described in the specification
  Arg (32)..(32): Arg with the chemical modification described in the specification

SEQ ID NO: 31 - protein, 34 aa, Artificial Sequence; identical to SEQ ID NO: 8
  Cyclic PYY Peptide Compound
  Ile (1)..(1): Ile with the chemical modification described in the specification
  Lys (28)..(28): Lys with the chemical modification described in the specification
  Cys (29)..(29): Cys, wherein the cys is a homocysteine with the chemical modification described in the specification
  Arg (33)..(33): Arg with the chemical modification described in the specification

SEQ ID NO: 32 - protein, 34 aa, Artificial Sequence; identical to SEQ ID NO: 21
  Cyclic PYY Peptide Compound
  Ile (1)..(1): Ile with the chemical modification described in the specification
  Lys (28)..(28): Lys with the chemical modification described in the specification
  Cys (29)..(29): Cys, wherein the cys is a homocysteine with the chemical modification described in the specification
  Arg (33)..(33): Arg with the chemical modification described in the specification

SEQ ID NO: 33 - protein, 34 aa, Artificial Sequence; identical to SEQ ID NO: 8
  Cyclic PYY Peptide Compound
  Ile (1)..(1): Ile with the chemical modification described in the specification
  Lys (28)..(28): Lys with the chemical modification described in the specification
  Cys (29)..(29): Cys, wherein the cys is a homocysteine with the chemical modification described in the specification
  Gln (32)..(32): Gln with the chemical modification described in the specification
  Arg (33)..(33): Arg with the chemical modification described in the specification

SEQ ID NO: 34 - protein, 33 aa, Artificial Sequence; identical to SEQ ID NO: 15
  Cyclic PYY Peptide Compound
  Lys (1)..(1): Lys with the chemical modification described in the specification
  Lys (27)..(27): Lys with the chemical modification described in the specification
  Cys (28)..(28): Cys with the chemical modification described in the specification
  Arg (32)..(32): Arg with the chemical modification described in the specification

SEQ ID NO: 35 - protein, 34 aa, Artificial Sequence; identical to SEQ ID NO: 8
  Cyclic PYY Peptide Compound
  Ile (1)..(1): Ile with the chemical modification described in the specification
  Lys (28)..(28): Lys with the chemical modification described in the specification
  Cys (29)..(29): Cys, wherein the cys is a homocysteine with the chemical modification described in the specification
  Arg (33)..(33): Arg with the chemical modification described in the specification

SEQ ID NO: 36 - protein, 33 aa, Artificial Sequence; identical to SEQ ID NO: 15
  Cyclic PYY Peptide Compound
  Lys (1)..(1): Lys with the chemical modification described in the specification
  Lys (27)..(27): Lys with the chemical modification described in the specification
  Cys (28)..(28): Cys, wherein the cys is a homocysteine with the chemical modification described in the specification
  Arg (32)..(32): Arg with the chemical modification described in the specification

SEQ ID NO: 37 - protein, 34 aa, Artificial Sequence; identical to SEQ ID NO: 8
  Cyclic PYY Peptide Compound
  Ile (1)..(1): Ile with the chemical modification described in the specification
  Lys (28)..(28): Lys with the chemical modification described in the specification
  Cys (29)..(29): Cys with the chemical modification described in the specification
  Arg (33)..(33): Arg with the chemical modification described in the specification

SEQ ID NO: 38 - protein, 34 aa, Artificial Sequence; identical to SEQ ID NO: 8
  Cyclic PYY Peptide Compound
  Ile (1)..(1): Ile with the chemical modification described in the specification
  Lys (28)..(28): Lys with the chemical modification described in the specification
  Cys (29)..(29): Cys, wherein the cys is a homocysteine with the chemical modification described in the specification
  Arg (33)..(33): Arg with the chemical modification described in the specification

SEQ ID NO: 39 - protein, 34 aa, Artificial Sequence
  Cyclic PYY Peptide Compound
  Ile (1)..(1): Ile with the chemical modification described in the specification
  Lys (28)..(28): Lys with the chemical modification described in the specification
  Cys (29)..(29): Cys, wherein the cys is a homocysteine with the chemical modification described in the specification
  Arg (33)..(33): Arg with the chemical modification described in the specification
ISPEAPGEDASPEELNRYYASLRHYLNKCTRQRY

SEQ ID NO: 40 - protein, 34 aa, Artificial Sequence
  Cyclic PYY Peptide Compound
  Ile (1)..(1): Ile with the chemical modification described in the specification
  Lys (28)..(28): Lys with the chemical modification described in the specification
  Leu (29)..(29): Leu, wherein the leu is a norleucine with the chemical modification described in the specification
  Arg (33)..(33): Arg with the chemical modification described in the specification
IKPEAPGEDASPEELNRYYASLRHYLNKLTRQRY

SEQ ID NO: 41 - protein, 34 aa, Artificial Sequence; identical to SEQ ID NO: 40
  Cyclic PYY Peptide Compound
  Ile (1)..(1): Ile with the chemical modification described in the specification
  Lys (28)..(28): Lys with the chemical modification described in the specification
  Leu (29)..(29): Leu, wherein the leu is a norleucine with the chemical modification described in the specification
  Arg (33)..(33): Arg with the chemical modification described in the specification

SEQ ID NO: 42 - protein, 34 aa, Artificial Sequence; identical to SEQ ID NO: 40
  Cyclic PYY Peptide Compound
  Ile (1)..(1): Ile with the chemical modification described in the specification
  Lys (28)..(28): Lys with the chemical modification described in the specification
  Leu (29)..(29): Leu, wherein the leu is a norleucine with the chemical modification described in the specification
  Arg (33)..(33): Arg with the chemical modification described in the specification

SEQ ID NO: 43 - protein, 34 aa, Artificial Sequence; identical to SEQ ID NO: 8
  Cyclic PYY Peptide Compound
  Ile (1)..(1): Ile with the chemical modification described in the specification
  Lys (28)..(28): Lys with the chemical modification described in the specification
  Cys (29)..(29): Cys, wherein the cys is a homocysteine with the chemical modification described in the specification
  Arg (33)..(33): Arg with the chemical modification described in the specification

SEQ ID NO: 44 - protein, 34 aa, Artificial Sequence; identical to SEQ ID NO: 4
  Cyclic PYY Peptide Compound
  Ile (1)..(1): Ile with the chemical modification described in the specification
  Lys (9)..(9): Lys with the chemical modification described in the specification
  Cys (29)..(29): Cys, wherein the cys is a homocysteine with the chemical modification described in the specification
  Arg (33)..(33): Arg with the chemical modification described in the specification

SEQ ID NO: 45 - protein, 34 aa, Artificial Sequence; identical to SEQ ID NO: 4
  Cyclic PYY Peptide Compound
  Ile (1)..(1): Ile with the chemical modification described in the specification
  Lys (9)..(9): Lys with the chemical modification described in the specification
  Cys (29)..(29): Cys, wherein the cys is a homocysteine with the chemical modification described in the specification
  Arg (33)..(33): Arg with the chemical modification described in the specification

SEQ ID NO: 46 - protein, 34 aa, Artificial Sequence; identical to SEQ ID NO: 8
  Cyclic PYY Peptide Compound
  Ile (1)..(1): Ile with the chemical modification described in the specification
  Lys (28)..(28): Lys with the chemical modification described in the specification
  Cys (29)..(29): Cys, wherein the cys is a homocysteine with the chemical modification described in the specification
  Arg (33)..(33): Arg with the chemical modification described in the specification

SEQ ID NO: 47 - protein, 34 aa, Artificial Sequence
  Cyclic PYY Peptide Compound
  Ile (1)..(1): Ile with the chemical modification described in the specification
  Lys (5)..(5): Lys with the chemical modification described in the specification
  Cys (29)..(29): Cys, wherein the cys is a homocysteine with the chemical modification described in the specification
  Arg (33)..(33): Arg with the chemical modification described in the specification
IKPEKPGEDASPEELNRYYASLRHYLNLCTRQRY

SEQ ID NO: 48 - protein, 34 aa, Artificial Sequence
  Cyclic PYY Peptide Compound
  Ile (1)..(1): Ile with the chemical modification described in the specification
  Lys (20)..(20): Lys with the chemical modification described in the specification
  Cys (29)..(29): Cys, wherein the cys is a homocysteine with the chemical modification described in the specification
  Arg (33)..(33): Arg with the chemical modification described in the specification
IKPEAPGEDASPEELNRYYKSLRHYLNLCTRQRY

SEQ ID NO: 49 - protein, 34 aa, Artificial Sequence; identical to SEQ ID NO: 8
  Cyclic PYY Peptide Compound
  Ile (1)..(1): Ile with the chemical modification described in the specification
  Lys (28)..(28): Lys with the chemical modification described in the specification
  Cys (29)..(29): Cys, wherein the cys is a homocysteine with the chemical modification described in the specification
  Arg (33)..(33): Arg with the chemical modification described in the specification

SEQ ID NO: 50 - protein, 34 aa, Artificial Sequence
  Cyclic PYY Peptide Compound
  Ile (1)..(1): Ile with the chemical modification described in the specification
  Lys (21)..(21): Lys with the chemical modification described in the specification
  Cys (29)..(29): Cys, wherein the cys is a homocysteine with the chemical modification described in the specification
  Arg (33)..(33): Arg with the chemical modification described in the specification
IKPEAPGEDASPEELNRYYAKLRHYLNLCTRQRY

SEQ ID NO: 51 - protein, 34 aa, Artificial Sequence; identical to SEQ ID NO: 39
  Cyclic PYY Peptide Compound
  Ile (1)..(1): Ile with the chemical modification described in the specification
  Lys (28)..(28): Lys with the chemical modification described in the specification
  Cys (29)..(29): Cys, wherein the cys is a homocysteine with the chemical modification described in the specification
  Arg (33)..(33): Arg with the chemical modification described in the specification

SEQ ID NO: 52 - protein, 34 aa, Artificial Sequence; identical to SEQ ID NO: 4
  Cyclic PYY Peptide Compound
  Ile (1)..(1): Ile with the chemical modification described in the specification
  Lys (9)..(9): Lys with the chemical modification described in the specification
  Cys (29)..(29): Cys, wherein the cys is a homocysteine with the chemical modification described in the specification
  Arg (33)..(33): Cys, wherein the cys is a homocysteine with the chemical modification described in the specification

SEQ ID NO: 53 - protein, 34 aa, Artificial Sequence; identical to SEQ ID NO: 4
  Cyclic PYY Peptide Compound
  Ile (1)..(1): Ile with the chemical modification described in the specification
  Lys (9)..(9): Lys with the chemical modification described in the specification
  Cys (29)..(29): Cys, wherein the cys is a homocysteine with the chemical modification described in the specification
  Arg (33)..(33): Arg with the chemical modification described in the specification

SEQ ID NO: 54 - protein, 34 aa, Artificial Sequence; identical to SEQ ID NO: 4
  Cyclic PYY Peptide Compound
  Ile (1)..(1): Ile with the chemical modification described in the specification
  Lys (9)..(9): Lys with the chemical modification described in the specification
  Cys (29)..(29): Cys, wherein the cys is a homocysteine with the chemical modification described in the specification
  Arg (33)..(33): Arg with the chemical modification described in the specification

SEQ ID NO: 55 - protein, 34 aa, Artificial Sequence; identical to SEQ ID NO: 50
  Cyclic PYY Peptide Compound
  Ile (1)..(1): Ile with the chemical modification described in the specification
  Lys (21)..(21): Lys with the chemical modification described in the specification
  Cys (29)..(29): Cys, wherein the cys is a homocysteine with the chemical modification described in the specification
  Arg (33)..(33): Arg with the chemical modification described in the specification

SEQ ID NO: 56 - protein, 34 aa, Artificial Sequence; identical to SEQ ID NO: 8
  Cyclic PYY Peptide Compound
  Ile (1)..(1): Ile with the chemical modification described in the specification
  Lys (28)..(28): Lys with the chemical modification described in the specification
  Cys (29)..(29): Cys, wherein the cys is a homocysteine with the chemical modification described in the specification

SEQ ID NO: 57 - protein, 34 aa, Artificial Sequence; identical to SEQ ID NO: 8
  Cyclic PYY Peptide Compound
  Ile (1)..(1): Ile with the chemical modification described in the specification
  Lys (28)..(28): Lys with the chemical modification described in the specification
  Cys (29)..(29): Cys, wherein the cys is a homocysteine with the chemical modification described in the specification

SEQ ID NO: 58 - protein, 34 aa, Artificial Sequence; identical to SEQ ID NO: 8
  Cyclic PYY Peptide Compound
  Ile (1)..(1): Ile with the chemical modification described in the specification
  Lys (28)..(28): Lys with the chemical modification described in the specification
  Cys (29)..(29): Cys, wherein the cys is a homocysteine with the chemical modification described in the specification
  Arg (33)..(33): Arg with the chemical modification described in the specification

SEQ ID NO: 59 - protein, 34 aa, Artificial Sequence; identical to SEQ ID NO: 48
  Cyclic PYY Peptide Compound
  Ile (1)..(1): Ile with the chemical modification described in the specification
  Lys (20)..(20): Lys with the chemical modification described in the specification
  Cys (29)..(29): Cys, wherein the cys is a homocysteine with the chemical modification described in the specification
  Arg (33)..(33): Arg with the chemical modification described in the specification

SEQ ID NO: 60 - protein, 34 aa, Artificial Sequence; identical to SEQ ID NO: 47
  Cyclic PYY Peptide Compound
  Ile (1)..(1): Ile with the chemical modification described in the specification
  Lys (5)..(5): Lys with the chemical modification described in the specification
  Cys (29)..(29): Cys, wherein the cys is a homocysteine with the chemical modification described in the specification
  Arg (33)..(33): Arg with the chemical modification described in the specification

SEQ ID NO: 61 - protein, 34 aa, Artificial Sequence; identical to SEQ ID NO: 8
  Cyclic PYY Peptide Compound
  Ile (1)..(1): Ile with the chemical modification described in the specification
  Lys (28)..(28): Lys with the chemical modification described in the specification
  Cys (29)..(29): Cys, wherein the cys is a homocysteine with the chemical modification described in the specification
  Arg (33)..(33): Arg with the chemical modification described in the specification

SEQ ID NO: 62 - protein, 34 aa, Artificial Sequence; identical to SEQ ID NO: 8
  Cyclic PYY Peptide Compound
  Ile (1)..(1): Ile with the chemical modification described in the specification
  Lys (28)..(28): Lys with the chemical modification described in the specification
  Cys (29)..(29): Cys, wherein the cys is a homocysteine with the chemical modification described in the specification
  Arg (33)..(33): Arg with the chemical modification described in the specification

SEQ ID NO: 63 - protein, 34 aa, Artificial Sequence; identical to SEQ ID NO: 8
  Cyclic PYY Peptide Compound
  Ile (1)..(1): Ile with the chemical modification described in the specification
  Lys (28)..(28): Lys with the chemical modification described in the specification
  Cys (29)..(29): Cys, wherein the cys is a homocysteine with the chemical modification described in the specification
  Arg (33)..(33): Arg with the chemical modification described in the specification

SEQ ID NO: 64 - protein, 34 aa, Artificial Sequence; identical to SEQ ID NO: 8
  Cyclic PYY Peptide Compound
  Ile (1)..(1): Ile with the chemical modification described in the specification
  Lys (28)..(28): Lys with the chemical modification described in the specification
  Cys (29)..(29): Cys, wherein the cys is a homocysteine with the chemical modification described in the specification
  Arg (33)..(33): Arg with the chemical modification described in the specification

SEQ ID NO: 65 - protein, 34 aa, Artificial Sequence; identical to SEQ ID NO: 8
  Cyclic PYY Peptide Compound
  Ile (1)..(1): Ile with the chemical modification described in the specification
  Lys (28)..(28): Lys with the chemical modification described in the specification
  Cys (29)..(29): Cys, wherein the cys is a homocysteine with the chemical modification described in the specification
  Arg (33)..(33): Arg with the chemical modification described in the specification

SEQ ID NO: 66 - protein, 34 aa, Artificial Sequence; identical to SEQ ID NO: 8
  Cyclic PYY Peptide Compound
  Ile (1)..(1): Ile with the chemical modification described in the specification
  Lys (28)..(28): Lys with the chemical modification described in the specification
  Cys (29)..(29): Cys, wherein the cys is a homocysteine with the chemical modification described in the specification
  Arg (33)..(33): Arg with the chemical modification described in the specification

SEQ ID NO: 67 - protein, 34 aa, Artificial Sequence; identical to SEQ ID NO: 8
  Cyclic PYY Peptide Compound
  Ile (1)..(1): Ile with the chemical modification described in the specification
  Lys (28)..(28): Lys with the chemical modification described in the specification
  Cys (29)..(29): Cys, wherein the cys is a homocysteine with the chemical modification described in the specification
  Arg (33)..(33): Arg with the chemical modification described in the specification

SEQ ID NO: 68 - protein, 34 aa, Artificial Sequence
  Cyclic PYY Peptide Compound
  Ile (1)..(1): Ile with the chemical modification described in the specification
  Lys (9)..(9): Lys with the chemical modification described in the specification
  Cys (28)..(28): Cys with the chemical modification described in the specification
  Arg (33)..(33): Arg with the chemical modification described in the specification
IKPEAPGEKASPEELNRYYASLRHYLNCVTRQRY

SEQ ID NO: 69 - protein, 35 aa, Artificial Sequence
  Cyclic PYY Peptide Compound
  Gly (1)..(1): Gly with the chemical modification described in the specification
  Glu (30)..(30): Glu with the chemical modification described in the specification
  Arg (34)..(34): Arg with the chemical modification described in the specification
GISPEAPGEKASPEELNRYYASLRHYLNLETRQRY

SEQ ID NO: 70 - protein, 35 aa, Artificial Sequence
  Cyclic PYY Peptide Compound
  Gly (1)..(1): Gly with the chemical modification described in the specification
  Glu (29)..(29): Glu with the chemical modification described in the specification
  Arg (34)..(34): Arg with the chemical modification described in the specification
GISPEAPGEKASPEELNRYYASLRHYLNEVTRQRY

SEQ ID NO: 71 - protein, 35 aa, Artificial Sequence; identical to SEQ ID NO: 70
  Cyclic PYY Peptide Compound
  Gly (1)..(1): Gly with the chemical modification described in the specification
  Glu (29)..(29): Glu with the chemical modification described in the specification
  Arg (34)..(34): Arg with the chemical modification described in the specification

SEQ ID NO: 72 - protein, 35 aa, Artificial Sequence; identical to SEQ ID NO: 70
  Cyclic PYY Peptide Compound
  Gly (1)..(1): Gly with the chemical modification described in the specification
  Lys (10)..(10): Lys with the chemical modification described in the specification
  Glu (29)..(29): Glu with the chemical modification described in the specification
  Arg (34)..(34): Arg with the chemical modification described in the specification

SEQ ID NO: 73 - protein, 35 aa, Artificial Sequence; identical to SEQ ID NO: 1
  Cyclic PYY Peptide Compound
  Ala (1)..(1): Ala with the chemical modification described in the specification
  Lys (10)..(10): Lys with the chemical modification described in the specification
  Cys (30)..(30): Cys, wherein the cys is a homocysteine with the chemical modification described in the specification
  Arg (34)..(34): Arg with the chemical modification described in the specification

SEQ ID NO: 74 - protein, 35 aa, Artificial Sequence; identical to SEQ ID NO: 1
  Cyclic PYY Peptide Compound
  Ala (1)..(1): Ala with the chemical modification described in the specification
  Lys (10)..(10): Lys with the chemical modification described in the specification
  Cys (30)..(30): Cys, wherein the cys is a homocysteine with the chemical modification described in the specification
  Arg (34)..(34): Arg with the chemical modification described in the specification

SEQ ID NO: 75 - protein, 34 aa, Artificial Sequence; identical to SEQ ID NO: 4
  Cyclic PYY Peptide Compound
  Ile (1)..(1): Ile with the chemical modification described in the specification
  Lys (9)..(9): Lys with the chemical modification described in the specification
  Cys (29)..(29): Cys with the chemical modification described in the specification
  Arg (33)..(33): Arg with the chemical modification described in the specification

SEQ ID NO: 76 - protein, 35 aa, Artificial Sequence
  Cyclic PYY Peptide Compound
  Ala (1)..(1): Ala with the chemical modification described in the specification
  Lys (10)..(10): Lys with the chemical modification described in the specification
  Lys (29)..(29): Lys with the chemical modification described in the specification
  Cys (30)..(30): Cys, wherein the cys is a homocysteine with the chemical modification described in the specification
  Arg (34)..(34): Arg with the chemical modification described in the specification
AIKPEAPGEKASPEELNRYYASLRHYLNKCTRQRY

SEQ ID NO: 77 - protein, 35 aa, Artificial Sequence
  Cyclic PYY Peptide Compound
  Ala (1)..(1): Ala with the chemical modification described in the specification
  Lys (10)..(10): Lys with the chemical modification described in the specification
  Lys (19)..(19): Lys with the chemical modification described in the specification
  Cys (30)..(30): Cys, wherein the cys is a homocysteine with the chemical modification described in the specification
  Arg (34)..(34): Arg with the chemical modification described in the specification
AIKPEAPGEKASPEELNRKYASLRHYLNLCTRQRY

SEQ ID NO: 78 - protein, 35 aa, Artificial Sequence; identical to SEQ ID NO: 1
  Cyclic PYY Peptide Compound
  Ala (1)..(1): Ala with the chemical modification described in the specification
  Lys (10)..(10): Lys with the chemical modification described in the specification
  Cys (30)..(30): Cys, wherein the cys is a homocysteine with the chemical modification described in the specification
  Gln (33)..(33): Gln with the chemical modification described in the specification
  Arg (34)..(34): Arg with the chemical modification described in the specification

SEQ ID NO: 79 - protein, 35 aa, Artificial Sequence; identical to SEQ ID NO: 1
  Cyclic PYY Peptide Compound
  Ala (1)..(1): Ala with the chemical modification described in the specification
  Lys (10)..(10): Lys with the chemical modification described in the specification
  Cys (30)..(30): Cys, wherein the cys is a homocysteine with the chemical modification described in the specification
  Arg (34)..(34): Arg with the chemical modification described in the specification

SEQ ID NO: 80 - protein, 35 aa, Artificial Sequence
  Cyclic PYY Peptide Compound
  Ala (1)..(1): Ala with the chemical modification described in the specification
  Lys (10)..(10): Lys with the chemical modification described in the specification
  Cys (30)..(30): Cys, wherein the cys is a homocysteine with the chemical modification described in the specification
  Arg (34)..(34): Arg with the chemical modification described in the specification
AIRPEAPGEKASPEELNRYYASLRHYLNWCTRQRY

SEQ ID NO: 81 - protein, 34 aa, Artificial Sequence
  Cyclic PYY Peptide Compound
  Ile (1)..(1): Ile with the chemical modification described in the specification
  Lys (9)..(9): Lys with the chemical modification described in the specification
  Cys (29)..(29): Cys with the chemical modification described in the specification
  Arg (33)..(33): Arg with the chemical modification described in the specification
IRPEAPGEKASPEELNRYYASLRHYLNWCTRQRY

SEQ ID NO: 82 - protein, 33 aa, Artificial Sequence
  Cyclic PYY Peptide Compound
  Lys (1)..(1): Lys with the chemical modification described in the specification
  Lys (8)..(8): Lys with the chemical modification described in the specification
  Cys (28)..(28): Cys with the chemical modification described in the specification
  Arg (32)..(32): Arg with the chemical modification described in the specification
KPEAPGEKASPEELNRYYASLRHYLNLCTRQRY

SEQ ID NO: 83 - protein, 35 aa, Artificial Sequence
  Cyclic PYY Peptide Compound
  Ile (1)..(1): Ile with the chemical modification described in the specification
  Lys (9)..(9): Lys with the chemical modification described in the specification
  Leu (29)..(29): Leu, wherein the leu is a norleucine with the chemical modification described in the specification
  Arg (33)..(33): Arg with the chemical modification described in the specification
IKPEAPGEKASPEELNRYYASLRHYLNLLVTRQRY

SEQ ID NO: 84 - protein, 35 aa, Artificial Sequence
  Cyclic PYY Peptide Compound
  Ile (1)..(1): Ile with the chemical modification described in the specification
  Lys (9)..(9): Lys with the chemical modification described in the specification
  Cys (29)..(29): Cys, wherein the cys is a homocysteine with the chemical modification described in the specification
  Arg (33)..(33): Arg with the chemical modification described in the specification
IKPEAPGEKASPEELNRYYASLRHYLNLCVTRQRY

SEQ ID NO: 85 - protein, 36 aa, Artificial Sequence
  Cyclic PYY Peptide Compound
  Ala (1)..(1): Ala with the chemical modification described in the specification
  Lys (22)..(22): Lys with the chemical modification described in the specification
  Cys (30)..(30): Cys, wherein the cys is a homocysteine with the chemical modification described in the specification
  Arg (34)..(34): Arg with the chemical modification described in the specification
AIKPEAPGEDASPEELNRYYAKLRHYLNLCVTRQRY

SEQ ID NO: 86 - protein, 36 aa, Artificial Sequence
  Cyclic PYY Peptide Compound
  Ala (1)..(1): Ala with the chemical modification described in the specification
  Lys (21)..(21): Lys with the chemical modification described in the specification
  Cys (30)..(30): Cys, wherein the cys is a homocysteine with the chemical modification described in the specification
  Arg (34)..(34): Arg with the chemical modification described in the specification
AIKPEAPGEDASPEELNRYYKSLRHYLNLCVTRQRY

SEQ ID NO: 87 - protein, 36 aa, Artificial Sequence
  Cyclic PYY Peptide Compound
  Ala (1)..(1): Ala with the chemical modification described in the specification
  Lys (6)..(6): Lys with the chemical modification described in the specification
  Cys (30)..(30): Cys, wherein the cys is a homocysteine with the chemical modification described in the specification
  Arg (34)..(34): Arg with the chemical modification described in the specification
AIKPEKPGEDASPEELNRYYASLRHYLNLCVTRQRY

SEQ ID NO: 88 - protein, 35 aa, Artificial Sequence
  Cyclic PYY Peptide Compound
  Gly (1)..(1): Gly with the chemical modification described in the specification
  Lys (10)..(10): Lys with the chemical modification described in the specification
  Cys (29)..(29): Cys with the chemical modification described in the specification
  Arg (34)..(34): Arg with the chemical modification described in the specification
GIKPEAPGEKASPEELNRYYASLRHYLNCVTRQRY

SEQ ID NO: 89 - protein, 35 aa, Artificial Sequence; identical to SEQ ID NO: 88
  Cyclic PYY Peptide Compound
  Gly (1)..(1): Gly with the chemical modification described in the specification
  Lys (10)..(10): Lys with the chemical modification described in the specification
  Cys (29)..(29): Cys with the chemical modification described in the specification
  Arg (34)..(34): Arg with the chemical modification described in the specification

SEQ ID NO: 90 - protein, 35 aa, Artificial Sequence
  Cyclic PYY Peptide Compound
  Ala (1)..(1): Ala with the chemical modification described in the specification
  Lys (10)..(10): Lys with the chemical modification described in the specification
  Cys (29)..(29): Cys with the chemical modification described in the specification
  Arg (34)..(34): Arg with the chemical modification described in the specification
AIKPEAPGEKASPEELNRYYASLRHYLNCVTRQRY

SEQ ID NO: 91 - protein, 35 aa, Artificial Sequence; identical to SEQ ID NO: 88
  Cyclic PYY Peptide Compound
  Gly (1)..(1): Gly with the chemical modification described in the specification
  Lys (10)..(10): Lys with the chemical modification described in the specification
  Cys (29)..(29): Cys, wherein the cys is a homocysteine with the chemical modification described in the specification
  Arg (34)..(34): Arg with the chemical modification described in the specification

SEQ ID NO: 92 - protein, 35 aa, Artificial Sequence; identical to SEQ ID NO: 1
  Cyclic PYY Peptide Compound
  Ala (1)..(1): Ala with the chemical modification described in the specification
  Lys (10)..(10): Lys with the chemical modification described in the specification
  Cys (30)..(30): Cys, wherein the cys is a homocysteine with the chemical modification described in the specification
  Arg (34)..(34): Arg with the chemical modification described in the specification

SEQ ID NO: 93 - protein, 35 aa, Artificial Sequence; identical to SEQ ID NO: 88
  Cyclic PYY Peptide Compound
  Gly (1)..(1): Gly with the chemical modification described in the specification
  Lys (10)..(10): Lys with the chemical modification described in the specification
  Cys (29)..(29): Cys, wherein the cys is a homocysteine with the chemical modification described in the specification
  Arg (34)..(34): Arg with the chemical modification described in the specification

SEQ ID NO: 94 - protein, 35 aa, Artificial Sequence; identical to SEQ ID NO: 90
  Cyclic PYY Peptide Compound
  Ala (1)..(1): Ala with the chemical modification described in the specification
  Lys (10)..(10): Lys with the chemical modification described in the specification
  Cys (29)..(29): Cys with the chemical modification described in the specification
  Arg (34)..(34): Arg with the chemical modification described in the specification

SEQ ID NO: 95 - protein, 35 aa, Artificial Sequence; identical to SEQ ID NO: 70
  Cyclic PYY Peptide Compound
  Gly (1)..(1): Gly with the chemical modification described in the specification
  Lys (10)..(10): Lys with the chemical modification described in the specification
  Glu (29)..(29): Glu with the chemical modification described in the specification
  Arg (34)..(34): Arg with the chemical modification described in the specification

SEQ ID NO: 96 - protein, 35 aa, Artificial Sequence; identical to SEQ ID NO: 1
  Cyclic PYY Peptide Compound
  Ala (1)..(1): Ala with the chemical modification described in the specification
  Lys (10)..(10): Lys with the chemical modification described in the specification
  Cys (30)..(30): Cys, wherein the cys is a homocysteine with the chemical modification described in the specification
  Arg (34)..(34): Arg with the chemical modification described in the specification

SEQ ID NO: 97 - protein, 35 aa, Artificial Sequence
  Cyclic PYY Peptide Compound
  Gly (1)..(1): Gly with the chemical modification described in the specification
  Lys (10)..(10): Lys with the chemical modification described in the specification
  Cys (30)..(30): Cys, wherein the cys is a homocysteine with the chemical modification described in the specification
  Arg (34)..(34): Arg with the chemical modification described in the specification
GIKPEAPGEKASPEELNRYYASLRHYLNLCTRQRY

SEQ ID NO: 98 - protein, 35 aa, Artificial Sequence
  Cyclic PYY Peptide Compound
  Gly (1)..(1): Gly with the chemical modification described in the specification
  Lys (10)..(10): Lys with the chemical modification described in the specification
  Cys (29)..(29): Cys with the chemical modification described in the specification
  Arg (34)..(34): Arg with the chemical modification described in the specification
GISPEAPGEKASPEELNRYYASLRHYLNCVTRQRY

SEQ ID NO: 99 - protein, 35 aa, Artificial Sequence; identical to SEQ ID NO: 90
  Cyclic PYY Peptide Compound
  Ala (1)..(1): Ala with the chemical modification described in the specification
  Lys (10)..(10): Lys with the chemical modification described in the specification
  Cys (29)..(29): Cys with the chemical modification described in the specification
  Arg (34)..(34): Arg with the chemical modification described in the specification

SEQ ID NO: 100 - protein, 35 aa, Artificial Sequence; identical to SEQ ID NO: 90
  Cyclic PYY Peptide Compound
  Ala (1)..(1): Ala with the chemical modification described in the specification
  Lys (10)..(10): Lys with the chemical modification described in the specification
  Cys (29)..(29): Cys with the chemical modification described in the specification
  Arg (34)..(34): Arg with the chemical modification described in the specification

SEQ ID NO: 101 - protein, 34 aa, Homo sapiens
IKPEAPGEDASPEELNRYYASLRHYLNLVTRQRY

SEQ ID NO: 102 - protein, 35 aa, Artificial Sequence; identical to SEQ ID NO: 1
  Conjugate 1
  Ala (1)..(1): Ala with the chemical modification described in the specification
  Lys (10)..(10): Lys with the chemical modification described in the specification
  Cys (29)..(29): Cys, wherein the cys is a homocysteine with the chemical modification described in the specification
  Arg (33)..(33): Arg with the chemical modification described in the specification

SEQ ID NO: 103 - protein, 35 aa, Artificial Sequence; identical to SEQ ID NO: 1
  Conjugate 2
  Ala (1)..(1): Ala with the chemical modification described in the specification
  Lys (10)..(10): Lys with the chemical modification described in the specification
  Cys (30)..(30): Cys, wherein the cys is a homocysteine with the chemical modification described in the specification
  Arg (34)..(34): Arg with the chemical modification described in the specification

SEQ ID NO: 104 - protein, 35 aa, Artificial Sequence; identical to SEQ ID NO: 1
  Conjugate 3
  Ala (1)..(1): Ala with the chemical modification described in the specification
  Lys (10)..(10): Lys with the chemical modification described in the specification
  Cys (30)..(30): Cys, wherein the cys is a homocysteine with the chemical modification described in the specification
  Arg (34)..(34): Arg with the chemical modification described in the specification

SEQ ID NO: 105 - protein, 34 aa, Artificial Sequence; identical to SEQ ID NO: 4
  Conjugate 4
  Ile (1)..(1): Ile with the chemical modification described in the specification
  Lys (9)..(9): Lys with the chemical modification described in the specification
  Cys (29)..(29): Cys with the chemical modification described in the specification
  Arg (33)..(33): Arg with the chemical modification described in the specification

SEQ ID NO: 106 - protein, 35 aa, Artificial Sequence; identical to SEQ ID NO: 76
  Conjugate 5
  Ala (1)..(1): Ala with the chemical modification described in the specification
  Lys (10)..(10): Lys with the chemical modification described in the specification
  Lys (29)..(29): Lys with the chemical modification described in the specification
  Cys (30)..(30): Cys, wherein the cys is a homocysteine with the chemical modification described in the specification
  Arg (34)..(34): Arg with the chemical modification described in the specification

SEQ ID NO: 107 - protein, 35 aa, Artificial Sequence; identical to SEQ ID NO: 77
  Conjugate 6
  Ala (1)..(1): Ala with the chemical modification described in the specification
  Lys (10)..(10): Lys with the chemical modification described in the specification
  Lys (19)..(19): Lys with the chemical modification described in the specification
  Cys (30)..(30): Cys, wherein the cys is a homocysteine with the chemical modification described in the specification
  Arg (34)..(34): Arg with the chemical modification described in the specification

SEQ ID NO: 108 - protein, 35 aa, Artificial Sequence; identical to SEQ ID NO: 1
  Conjugate 7
  Ala (1)..(1): Ala with the chemical modification described in the specification
  Lys (10)..(10): Lys with the chemical modification described in the specification
  Cys (30)..(30): Cys, wherein the cys is a homocysteine with the chemical modification described in the specification
  Gln (33)..(33): Gln with the chemical modification described in the specification
  Arg (34)..(34): Arg with the chemical modification described in the specification

SEQ ID NO: 109 - protein, 35 aa, Artificial Sequence; identical to SEQ ID NO: 1
  Conjugate 8
  Ala (1)..(1): Ala with the chemical modification described in the specification
  Lys (10)..(10): Lys with the chemical modification described in the specification
  Cys (30)..(30): Cys, wherein the cys is a homocysteine with the chemical modification described in the specification
  Arg (34)..(34): Arg with the chemical modification described in the specification

SEQ ID NO: 110 - protein, 35 aa, Artificial Sequence; identical to SEQ ID NO: 80
  Conjugate 9
  Ala (1)..(1): Ala with the chemical modification described in the specification
  Lys (10)..(10): Lys with the chemical modification described in the specification
  Cys (30)..(30): Cys, wherein the cys is a homocysteine with the chemical modification described in the specification
  Arg (34)..(34): Arg with the chemical modification described in the specification

SEQ ID NO: 111 - protein, 34 aa, Artificial Sequence; identical to SEQ ID NO: 81
  Conjugate 10
  Ile (1)..(1): Ile with the chemical modification described in the specification
  Lys (9)..(9): Lys with the chemical modification described in the specification
  Cys (29)..(29): Cys with the chemical modification described in the specification
  Arg (33)..(33): Arg with the chemical modification described in the specification

SEQ ID NO: 112 - protein, 33 aa, Artificial Sequence; identical to SEQ ID NO: 82
  Conjugate 11
  Lys (1)..(1): Lys with the chemical modification described in the specification
  Lys (8)..(8): Lys with the chemical modification described in the specification
  Cys (28)..(28): Cys with the chemical modification described in the specification
  Arg (32)..(32): Arg with the chemical modification described in the specification

SEQ ID NO: 113 - protein, 35 aa, Artificial Sequence; identical to SEQ ID NO: 83
  Conjugate 12
  Ile (1)..(1): Ile with the chemical modification described in the specification
  Lys (9)..(9): Lys with the chemical modification described in the specification
  Leu (29)..(29): Leu, wherein the leu is a norleucine with the chemical modification described in the specification
  Arg (33)..(33): Arg with the chemical modification described in the specification

SEQ ID NO: 114 - protein, 35 aa, Artificial Sequence; identical to SEQ ID NO: 84
  Conjugate 13
  Ile (1)..(1): Ile with the chemical modification described in the specification
  Lys (10)..(10): Lys with the chemical modification described in the specification
  Cys (30)..(30): Cys, wherein the cys is a homocysteine with the chemical modification described in the specification
  Arg (34)..(34): Arg with the chemical modification described in the specification

SEQ ID NO: 115 - protein, 36 aa, Artificial Sequence; identical to SEQ ID NO: 85
  Conjugate 14
  Ala (1)..(1): Ala with the chemical modification described in the specification
  Lys (22)..(22): Lys with the chemical modification described in the specification
  Cys (30)..(30): Cys, wherein the cys is a homocysteine with the chemical modification described in the specification
  Arg (34)..(34): Arg with the chemical modification described in the specification

SEQ ID NO: 116 - protein, 36 aa, Artificial Sequence; identical to SEQ ID NO: 86
  Conjugate 15
  Ala (1)..(1): Ala with the chemical modification described in the specification
  Lys (21)..(21): Lys with the chemical modification described in the specification
  Cys (30)..(30): Cys, wherein the cys is a homocysteine with the chemical modification described in the specification
  Arg (34)..(34): Arg with the chemical modification described in the specification

SEQ ID NO: 117 - protein, 36 aa, Artificial Sequence; identical to SEQ ID NO: 87
  Conjugate 16
  Ala (1)..(1): Ala with the chemical modification described in the specification
  Lys (6)..(6): Lys with the chemical modification described in the specification
  Cys (30)..(30): Cys with the chemical modification described in the specification
  Arg (34)..(34): Arg with the chemical modification described in the specification

SEQ ID NO: 118 - protein, 35 aa, Artificial Sequence; identical to SEQ ID NO: 88
  Conjugate 17
  Gly (1)..(1): Gly with the chemical modification described in the specification
  Lys (10)..(10): Lys with the chemical modification described in the specification
  Cys (29)..(29): Cys with the chemical modification described in the specification
  Arg (34)..(34): Arg with the chemical modification described in the specification

SEQ ID NO: 119 - protein, 35 aa, Artificial Sequence; identical to SEQ ID NO: 88
  Conjugate 18
  Gly (1)..(1): Gly with the chemical modification described in the specification
  Lys (10)..(10): Lys with the chemical modification described in the specification
  Cys (29)..(29): Cys with the chemical modification described in the specification
  Arg (34)..(34): Arg with the chemical modification described in the specification

SEQ ID NO: 120 - protein, 35 aa, Artificial Sequence; identical to SEQ ID NO: 90
  Conjugate 19
  Ala (1)..(1): Ala with the chemical modification described in the specification
  Lys (10)..(10): Lys with the chemical modification described in the specification
  Cys (29)..(29): Cys with the chemical modification described in the specification
  Arg (34)..(34): Arg with the chemical modification described in the specification

SEQ ID NO: 121 - protein, 35 aa, Artificial Sequence; identical to SEQ ID NO: 88
  Conjugate 20
  Gly (1)..(1): Gly with the chemical modification described in the specification
  Lys (10)..(10): Lys with the chemical modification described in the specification
  Cys (29)..(29): Cys, wherein the cys is a homocysteine with the chemical modification described in the specification
  Arg (34)..(34): Arg with the chemical modification described in the specification

SEQ ID NO: 122 - protein, 35 aa, Artificial Sequence; identical to SEQ ID NO: 1
  Conjugate 21
  Ala (1)..(1): Ala with the chemical modification described in the specification
  Lys (10)..(10): Lys with the chemical modification described in the specification
  Cys (30)..(30): Cys with the chemical modification described in the specification
  Arg (34)..(34): Arg with the chemical modification described in the specification

SEQ ID NO: 123 - protein, 35 aa, Artificial Sequence; identical to SEQ ID NO: 88
  Conjugate 22
  Gly (1)..(1): Gly with the chemical modification described in the specification
  Lys (10)..(10): Lys with the chemical modification described in the specification
  Cys (29)..(29): Cys, wherein the cys is a homocysteine with the chemical modification described in the specification
  Arg (34)..(34): Arg with the chemical modification described in the specification

SEQ ID NO: 124 - protein, 35 aa, Artificial Sequence; identical to SEQ ID NO: 90
  Conjugate 23
  Ala (1)..(1): Ala with the chemical modification described in the specification
  Lys (10)..(10): Lys with the chemical modification described in the specification
  Cys (29)..(29): Cys with the chemical modification described in the specification
  Arg (34)..(34): Arg with the chemical modification described in the specification

SEQ ID NO: 125 - protein, 35 aa, Artificial Sequence; identical to SEQ ID NO: 70
  Conjugate 24
  Gly (1)..(1): Gly with the chemical modification described in the specification
  Lys (10)..(10): Lys with the chemical modification described in the specification
  Glu (29)..(29): Glu with the chemical modification described in the specification
  Arg (34)..(34): Arg with the chemical modification described in the specification

SEQ ID NO: 126 - protein, 35 aa, Artificial Sequence; identical to SEQ ID NO: 1
  Conjugate 25
  Ala (1)..(1): Ala with the chemical modification described in the specification
  Lys (10)..(10): Lys with the chemical modification described in the specification
  Cys (30)..(30): Cys, wherein the cys is a homocysteine with the chemical modification described in the specification
  Arg (34)..(34): Arg with the chemical modification described in the specification

SEQ ID NO: 127 - protein, 35 aa, Artificial Sequence; identical to SEQ ID NO: 97
  Conjugate 26
  Gly (1)..(1): Gly with the chemical modification described in the specification
  Lys (10)..(10): Lys with the chemical modification described in the specification
  Cys (30)..(30): Cys, wherein the cys is a homocysteine with the chemical modification described in the specification
  Arg (34)..(34): Arg with the chemical modification described in the specification

SEQ ID NO: 128 - protein, 107 aa, Homo sapiens
EIVLTQSPATLSLSPGERATLSCRASQSVSSYLAWYQQKPGQAPRLLIYDASNRATGIPARFSGSGSGTDFTLTISSLEPEDFAVYYCQQRSNWPLTFGQGTKVEIK

SEQ ID NO: 129 - protein, 119 aa, Homo sapiens
EVQLLESGGGLVQPGGSLRLSCAASGFTFSSYAMSWVRQAPGKGLEWVSAISGSGGSTYYADSVKGRFTISRDNSKNTLYLQMNSLRAEDTAVYYCAKYDGIYGELDFWGQGTLVTVSS

SEQ ID NO: 130 - protein, 10 aa, Homo sapiens
YDGIYGELDF

SEQ ID NO: 131 - protein, 115 aa, Artificial Sequence
  concatenation of IGHV3-23*01 and IGHJ1*01
EVQLLESGGGLVQPGGSLRLSCAASGFTFSSYAMSWVRQAPGKGLEWVSAISGSGGSTYYADSVKGRFTISRDNSKNTLYLQMNSLRAEDTAVYYCAKAEYFQHWGQGTLVTVSS

SEQ ID NO: 132 - protein, 98 aa, Homo sapiens
EVQLLESGGGLVQPGGSLRLSCAASGFTFSSYAMSWVRQAPGKGLEWVSAISGSGGSTYYADSVKGRFTISRDNSKNTLYLQMNSLRAEDTAVYYCAK

SEQ ID NO: 133 - protein, 17 aa, Homo sapiens
AEYFQHWGQGTLVTVSS

SEQ ID NO: 134 - protein, 107 aa, Artificial Sequence
  concatenation of IGKV3-11*01 and IGKJ1*01
EIVLTQSPATLSLSPGERATLSCRASQSVSSYLAWYQQKPGQAPRLLIYDASNRATGIPARFSGSGSGTDFTLTISSLEPEDFAVYYCQQRSNWPWTFGQGTKVEIK

SEQ ID NO: 135 - protein, 95 aa, Homo sapiens
EIVLTQSPATLSLSPGERATLSCRASQSVSSYLAWYQQKPGQAPRLLIYDASNRATGIPARFSGSGSGTDFTLTISSLEPEDFAVYYCQQRSNWP

SEQ ID NO: 136 - protein, 12 aa, Homo sapiens
WTFGQGTKVEIK

SEQ ID NO: 137 - protein, 119 aa, Artificial Sequence
  MSCB97 VH
EVQLLESGGGLVQPGGSLRLSCAASGFTFSSYAMSWVRQAPGKGLEWVSAISGSGGSTYYADSVKGRFTISRDNSKNTLYLQMNSLRAEDTAVYYCAKYDGCYGELDFWGQGTLVTVSS

SEQ ID NO: 138 - protein, 446 aa, Artificial Sequence
  MSCB97 HC
EVQLLESGGGLVQPGGSLRLSCAASGFTFSSYAMSWVRQAPGKGLEWVSAISGSGGSTYYADSVKGRFTISRDNSKNTLYLQMNSLRAEDTAVYYCAKYDGCYGELDFWGQGTLVTVSSASTKGPSVFPLAPCSRSTSESTAALGCLVKDYFPEPVTVSWNSGALTSGVHTFPAVLQSSGLYSLSSVVTVPSSSLGTKTYTCNVDHKPSNTKVDKRVESKYGPPCPPCPAPEAAGGPSVFLFPPKPKDTLMISRTPEVTCVVVDVSQEDPEVQFNWYVDGVEVHNAKTKPREEQFNSTYRVVSVLTVLHQDWLNGKEYKCKVSNKGLPSSIEKTISKAKGQPREPQVYTLPPSQEEMTKNQVSLTCLVKGFYPSDIAVEWESNGQPENNYKTTPPVLDSDGSFFLYSRLTVDKSRWQEGNVFSCSVMHEALHNHYTQKSLSLSLGK

SEQ ID NO: 139 - protein, 107 aa, Artificial Sequence; identical to SEQ ID NO: 128
  MSCB97 VL

SEQ ID NO: 140 - protein, 214 aa, Artificial Sequence
  MSCB97 LC
EIVLTQSPATLSLSPGERATLSCRASQSVSSYLAWYQQKPGQAPRLLIYDASNRATGIPARFSGSGSGTDFTLTISSLEPEDFAVYYCQQRSNWPLTFGQGTKVEIKRTVAAPSVFIFPPSDEQLKSGTASVVCLLNNFYPREAKVQWKVDNALQSGNSQESVTEQDSKDSTYSLSSTLTLSKADYEKHKVYACEVTHQGLSSPVTKSFNRGEC

SEQ ID NO: 141 - protein, 5 aa, Artificial Sequence
  MSCB97 HCDR1
SYAMS

SEQ ID NO: 142 - protein, 17 aa, Artificial Sequence
  MSCB97 HCDR2
AISGSGGSTYYADSVKG

SEQ ID NO: 143 - protein, 10 aa, Artificial Sequence
  MSCB97 HCDR3
YDGCYGELDF

SEQ ID NO: 144 - protein, 11 aa, Artificial Sequence
  MSCB97 LCDR1
RASQSVSSYLA

SEQ ID NO: 145 - protein, 7 aa, Artificial Sequence
  MSCB97 LCDR2
DASNRAT

SEQ ID NO: 146 - protein, 9 aa, Artificial Sequence
  MSCB97 LCDR3
QQRSNWPLT

SEQ ID NO: 147 - protein, 35 aa, Artificial Sequence
  Cyclic PYY Peptide Compound
  Ala (1)..(1): Ala with chemical modification described in the specification
  Cys (30)..(30): Cys, wherein the cys is a homocysteine with chemical modification described in the specification
  Arg (34)..(34): Arg with chemical modification described in the specification
AIKPEAPGEDASPEELNRYYASLRHYLNLCTRQRY

SEQ ID NO: 148 - protein, 35 aa, Artificial Sequence; identical to SEQ ID NO: 1
  Cyclic PYY Peptide Compound
  Ala (1)..(1): Ala with chemical modification described in the specification
  Lys (10)..(10): Lys with chemical modification described in the specification
  Cys (30)..(30): Cys, wherein the cys is a homocysteine with chemical modification described in the specification
  Arg (34)..(34): Arg with chemical modification described in the specification

SEQ ID NO: 149 - protein, 35 aa, Artificial Sequence
  Cyclic PYY Peptide Compound
  Gly (1)..(1): Gly with chemical modification described in the specification
  Glu (29)..(29): Glu with chemical modification described in the specification
  Arg (34)..(34): Arg with chemical modification described in the specification
GIKPEAPGEDASPEELNRYYASLRHYLNEVTRQRY

SEQ ID NO: 150 - protein, 35 aa, Artificial Sequence
  Cyclic PYY Peptide Compound
  Gly (1)..(1): Gly with chemical modification described in the specification
  Lys (10)..(10): Lys with chemical modification described in the specification
  Glu (29)..(29): Glu with chemical modification described in the specification
  Arg (34)..(34): Arg with chemical modification described in the specification
GIKPEAPGEKASPEELNRYYASLRHYLNEVTRQRY

SEQ ID NO: 151 - protein, 35 aa, Artificial Sequence
  Cyclic PYY Peptide Compound
  Gly (1)..(1): Gly with chemical modification described in the specification
  Cys (29)..(29): Cys with chemical modification described in the specification
  Arg (34)..(34): Arg with chemical modification described in the specification
GIKPEAPGEDASPEELNRYYASLRHYLNCVTRQRY

SEQ ID NO: 152 - protein, 35 aa, Artificial Sequence; identical to SEQ ID NO: 88
  Cyclic PYY Peptide Compound
  Gly (1)..(1): Gly with chemical modification described in the specification
  Lys (10)..(10): Lys with chemical modification described in the specification
  Cys (29)..(29): Cys with chemical modification described in the specification
  Arg (34)..(34): Arg with chemical modification described in the specification

SEQ ID NO: 153 - protein, 35 aa, Artificial Sequence
  Cyclic PYY Peptide Compound
  Ala (1)..(1): Ala with chemical modification described in the specification
  Cys (29)..(29): Cys with chemical modification described in the specification
  Arg (34)..(34): Arg with chemical modification described in the specification
AIKPEAPGEDASPEELNRYYASLRHYLNCVTRQRY

SEQ ID NO: 154 - protein, 35 aa, Artificial Sequence; identical to SEQ ID NO: 90
  Cyclic PYY Peptide Compound
  Ala (1)..(1): Ala with chemical modification described in the specification
  Lys (10)..(10): Lys with chemical modification described in the specification
  Cys (29)..(29): Cys with chemical modification described in the specification
  Arg (34)..(34): Arg with chemical modification described in the specification

SEQ ID NO: 155 - protein, 35 aa, Artificial Sequence; identical to SEQ ID NO: 153
  Cyclic PYY Peptide Compound
  Ala (1)..(1): Ala with chemical modification described in the specification
  Cys (29)..(29): Cys with chemical modification described in the specification
  Arg (34)..(34): Arg with chemical modification described in the specification

SEQ ID NO: 156 - protein, 35 aa, Artificial Sequence; identical to SEQ ID NO: 90
  Cyclic PYY Peptide Compound
  Ala (1)..(1): Ala with chemical modification described in the specification
  Lys (10)..(10): Lys with chemical modification described in the specification
  Cys (29)..(29): Cys with chemical modification described in the specification
  Arg (34)..(34): Arg with chemical modification described in the specification